European Patent Specification EP 3 773 518 B1, published March 5, 2025. Title: Polymeric Materials And Articles manufactured There From. Applicant: The Procter & Gamble Company Williams, Christopher B. Zawaski, Callie E. Long, Timothy E. Pekkanen, Allison M. White, Benjamin T. Hodgdon, Travis K. Graham, Douglas M. Barnabas, Freddy A. Kenneally, Corey J. The sequence listing filed with the application follows.

SEQUENCE LISTING (1 sequence)

SEQ ID NO: 1 - protein, 773 aa, Bacillus sp.
AEGNTREDNFKHLLGNDNVKRPSEAGALQLQEVDGQMTLVDQHGEKIQLRGMSTHGLQWFPEILNDNAYKALANDWESNMIRLAMYVGENGYASNPELIKSRVIKGIDLAIENDMYVIVDWHVHAPGDPRDPVYAGAEDFFRDIAALYPNNPHIIYELANEPSSNNNGGAGIPNNEEGWNAVKEYADPIVEMLRDSGNADDNIIIVGSPNWSQRPDLAADNPINDHHTMYTVHFYTGSHAASTESYPPETPNSERGNVMSNTRYALENGVAVFATEWGTSQANGDGGPYFDEADVWIEFLNENNISWANWSLTNKNEVSGAFTPFELGKSNATNLDPGPDHVWAPEELSLSGEYVRARIKGVNYEPIDRTKYTKVLWDFNDGTKQGFGVNSDSPNKELIAVDNENNTLKVSGLDVSNDVSDGNFWANARLSADGWGKSVDILGAEKLTMDVIVDEPTTVAIAAIPQSSKSGWANPERAVRVNAEDFVQQTDGKYKAGLTITGEDAPNLKNIAFHEEDNNMNNIILFVGTDAADVIYLDNIKVIGTEVEIPVVHDPKGEAVLPSVFEDGTRQGWDWAGESGVKTALTIEEANGSNALSWEFGYPEVKPSDNWATAPRLDFWKSDLVRGENDYVAFDFYLDPVRATEGAMNINLVFQPPTNGYWVQAPKTYTINFDELEEANQVNGLYHYEVKINVRDITNIQDDTLLRNMMIIFADVESDFAGRVFVDNVRFEGAATTEPVEPEPVDPGEETPPVDEKEAKKEQKEAEKEEKEE